European Patent Application EP 4 755 905 A1, published June 10, 2026. Title: TRUNCATED PROGRANULIN PROTEIN AND USES THEREOF. Applicant: Fraunhofer-Gesellschaft zur Förderung der angewandten Forschung e.V. Application EP, filed December 5, 2024. The sequence listing filed with the application follows.

SEQUENCE LISTING (15 sequences)

SEQ ID NO: 1 - protein, 593 aa, Homo sapiens
MWTLVSWVALTAGLVAGTRCPDGQFCPVACCLDPGGASYSCCRPLLDKWPTTLSRHLGGPCQVDAHCSAGHSCIFTVSGTSSCCPFPEAVACGDGHHCCPRGFHCSADGRSCFQRSGNNSVGAIQCPDSQFECPDFSTCCVMVDGSWGCCPMPQASCCEDRVHCCPHGAFCDLVHTRCITPTGTHPLAKKLPAQRTNRAVALSSSVMCPDARSRCPDGSTCCELPSGKYGCCPMPNATCCSDHLHCCPQDTVCDLIQSKCLSKENATTDLLTKLPAHTVGDVKCDMEVSCPDGYTCCRLQSGAWGCCPFTQAVCCEDHIHCCPAGFTCDTQKGTCEQGPHQVPWMEKAPAHLSLPDPQALKRDVPCDNVSSCPSSDTCCQLTSGEWGCCPIPEAVCCSDHQHCCPQGYTCVAEGQCQRGSEIVAGLEKMPARRASLSHPRDIGCDQHTSCPVGQTCCPSLGGSWACCQLPHAVCCEDRQHCCPAGYTCNVKARSCEKEVVSAQPATFLARSPHVGVKDVECGEGHFCHDNQTCCRDNRQGWACCPYRQGVCCADRRHCCPAGFRCAARGTKCLRREAPRWDAPLRDPALRQLL

SEQ ID NO: 2 - protein, 152 aa, synthetic construct
  source 1..152: note = Domain 6, 7 and unstructured C-terminus of PGRN
IGCDQHTSCPVGQTCCPSLGGSWACCQLPHAVCCEDRQHCCPAGYTCNVKARSCEKEVVSAQPATFLARSPHVGVKDVECGEGHFCHDNQTCCRDNRQGWACCPYRQGVCCADRRHCCPAGFRCAARGTKCLRREAPRWDAPLRDPALRQLL

SEQ ID NO: 3 - protein, 76 aa, synthetic construct
  source 1..76: note = Domain 7 and unstructured C-terminus of PGRN
DVECGEGHFCHDNQTCCRDNRQGWACCPYRQGVCCADRRHCCPAGFRCAARGTKCLRREAPRWDAPLRDPALRQLL

SEQ ID NO: 4 - protein, 19 aa, synthetic construct
  source 1..19: note = Signal peptide
MYRMQLLSCIALSLALVTN

SEQ ID NO: 5 - protein, 30 aa, synthetic construct
  source 1..30: note = TwinStrep-Tag
WSHPQFEKGGGSGGGSGGSAWSHPQFEKDI

SEQ ID NO: 6 - protein, 6 aa, synthetic construct
  source 1..6: note = Linker
GSGSGS

SEQ ID NO: 7 - protein, 237 aa, synthetic construct
  source 1..237: note = mCherry (Mock)
VSKGEEDNMAIIKEFMRFKVHMEGSVNGHEFEIEGEGEGRPYEGTQTAKLKVTKGGPLPFAWDILSPQFMYGSKAYVKHPADIPDYLKLSFPEGFNWERVMNFEDGGVVTVTQDSSLQDGEFIYKVKLRGTNFPSDGPVMQCRTMGWEASTERMYPEDGALKGEIKQRLKLKDGGHYDAEVKTTYKAKKPVQLPGAYNVDIKLDILSHNEDYTIVEQYERAEGRHSTGGMDELYKDI

SEQ ID NO: 8 - protein, 451 aa, synthetic construct
  source 1..451: note = Construct 16 (C16) (Figure 1 B)
MYRMQLLSCIALSLALVTNSWSHPQFEKGGGSGGGSGGSAWSHPQFEKDIGSGSGSVSKGEEDNMAIIKEFMRFKVHMEGSVNGHEFEIEGEGEGRPYEGTQTAKLKVTKGGPLPFAWDILSPQFMYGSKAYVKHPADIPDYLKLSFPEGFNWERVMNFEDGGVVTVTQDSSLQDGEFIYKVKLRGTNFPSDGPVMQCRTMGWEASTERMYPEDGALKGEIKQRLKLKDGGHYDAEVKTTYKAKKPVQLPGAYNVDIKLDILSHNEDYTIVEQYERAEGRHSTGGMDELYKDIGSGSGSIGCDQHTSCPVGQTCCPSLGGSWACCQLPHAVCCEDRQHCCPAGYTCNVKARSCEKEVVSAQPATFLARSPHVGVKDVECGEGHFCHDNQTCCRDNRQGWACCPYRQGVCCADRRHCCPAGFRCAARGTKCLRREAPRWDAPLRDPALRQLL

SEQ ID NO: 9 - protein, 293 aa, synthetic construct
  source 1..293: note = Construct 18 (C18) (Figure 1 B)
MYRMQLLSCIALSLALVTNSWSHPQFEKGGGSGGGSGGSAWSHPQFEKDIGSGSGSVSKGEEDNMAIIKEFMRFKVHMEGSVNGHEFEIEGEGEGRPYEGTQTAKLKVTKGGPLPFAWDILSPQFMYGSKAYVKHPADIPDYLKLSFPEGFNWERVMNFEDGGVVTVTQDSSLQDGEFIYKVKLRGTNFPSDGPVMQCRTMGWEASTERMYPEDGALKGEIKQRLKLKDGGHYDAEVKTTYKAKKPVQLPGAYNVDIKLDILSHNEDYTIVEQYERAEGRHSTGGMDELYKDI

SEQ ID NO: 10 - protein, 319 aa, synthetic construct
  source 1..319: note = Construct 19 (C19) (Figure 1 B)
MYRMQLLSCIALSLALVTNSWSHPQFEKGGGSGGGSGGSAWSHPQFEKDIGSGSGSVSKGEEDNMAIIKEFMRFKVHMEGSVNGHEFEIEGEGEGRPYEGTQTAKLKVTKGGPLPFAWDILSPQFMYGSKAYVKHPADIPDYLKLSFPEGFNWERVMNFEDGGVVTVTQDSSLQDGEFIYKVKLRGTNFPSDGPVMQCRTMGWEASTERMYPEDGALKGEIKQRLKLKDGGHYDAEVKTTYKAKKPVQLPGAYNVDIKLDILSHNEDYTIVEQYERAEGRHSTGGMDELYKDIGSGSGSRREAPRWDAPLRDPALRQLL

SEQ ID NO: 11 - protein, 375 aa, synthetic construct
  source 1..375: note = Construct 20 (C20) (Figure 1 B)
MYRMQLLSCIALSLALVTNSWSHPQFEKGGGSGGGSGGSAWSHPQFEKDIGSGSGSVSKGEEDNMAIIKEFMRFKVHMEGSVNGHEFEIEGEGEGRPYEGTQTAKLKVTKGGPLPFAWDILSPQFMYGSKAYVKHPADIPDYLKLSFPEGFNWERVMNFEDGGVVTVTQDSSLQDGEFIYKVKLRGTNFPSDGPVMQCRTMGWEASTERMYPEDGALKGEIKQRLKLKDGGHYDAEVKTTYKAKKPVQLPGAYNVDIKLDILSHNEDYTIVEQYERAEGRHSTGGMDELYKDIGSGSGSDVECGEGHFCHDNQTCCRDNRQGWACCPYRQGVCCADRRHCCPAGFRCAARGTKCLRREAPRWDAPLRDPALRQLL

SEQ ID NO: 12 - protein, 449 aa, synthetic construct
  source 1..449: note = Siltuximab (DrugBank ID DB09036) Heavy Chain Sequence
EVQLVESGGKLLKPGGSLKLSCAASGFTFSSFAMSWFRQSPEKRLEWVAEISSGGSYTYYPDTVTGRFTISRDNAKNTLYLEMSSLRSEDTAMYYCARGLWGYYALDYWGQGTSVTVSSASTKGPSVFPLAPSSKSTSGGTAALGCLVKDYFPEPVTVSWNSGALTSGVHTFPAVLQSSGLYSLSSVVTVPSSSLGTQTYICNVNHKPSNTKVDKKVEPKSCDKTHTCPPCPAPELLGGPSVFLFPPKPKDTLMISRTPEVTCVVVDVSHEDPEVKFNWYVDGVEVHNAKTKPREEQYNSTYRVVSVLTVLHQDWLNGKEYKCKVSNKALPAPIEKTISKAKGQPREPQVYTLPPSRDELTKNQVSLTCLVKGFYPSDIAVEWESNGQPENNYKTTPPVLDSDGSFFLYSKLTVDKSRWQQGNVFSCSVMHEALHNHYTQKSLSLSPGK

SEQ ID NO: 13 - protein, 213 aa, synthetic construct
  source 1..213: note = Siltuximab (DrugBank ID DB09036) Light Chain Sequence
QIVLIQSPAIMSASPGEKVTMTCSASSSVSYMYWYQQKPGSSPRLLIYDTSNLASGVPVRFSGSGSGTSYSLTISRMEAEDAATYYCQQWSGYPYTFGGGTKLEIKRTVAAPSVFIFPPSDEQLKSGTASVVCLLNNFYPREAKVQWKVDNALQSGNSQESVTEQDSKDSTYSLSSTLTLSKADYEKHKVYACEVTHQGLSSPVTKSFNRGEC

SEQ ID NO: 14 - protein, 627 aa, synthetic construct
  source 1..627: note = Signal peptide_Siltuximab heavy chain_Linker_Domain 6, 7 and unstructured C-terminus of PGRN_fusion protein
MYRMQLLSCIALSLALVTNSEVQLVESGGKLLKPGGSLKLSCAASGFTFSSFAMSWFRQSPEKRLEWVAEISSGGSYTYYPDTVTGRFTISRDNAKNTLYLEMSSLRSEDTAMYYCARGLWGYYALDYWGQGTSVTVSSASTKGPSVFPLAPSSKSTSGGTAALGCLVKDYFPEPVTVSWNSGALTSGVHTFPAVLQSSGLYSLSSVVTVPSSSLGTQTYICNVNHKPSNTKVDKKVEPKSCDKTHTCPPCPAPELLGGPSVFLFPPKPKDTLMISRTPEVTCVVVDVSHEDPEVKFNWYVDGVEVHNAKTKPREEQYNSTYRVVSVLTVLHQDWLNGKEYKCKVSNKALPAPIEKTISKAKGQPREPQVYTLPPSRDELTKNQVSLTCLVKGFYPSDIAVEWESNGQPENNYKTTPPVLDSDGSFFLYSKLTVDKSRWQQGNVFSCSVMHEALHNHYTQKSLSLSPGKGSGSGSIGCDQHTSCPVGQTCCPSLGGSWACCQLPHAVCCEDRQHCCPAGYTCNVKARSCEKEVVSAQPATFLARSPHVGVKDVECGEGHFCHDNQTCCRDNRQGWACCPYRQGVCCADRRHCCPAGFRCAARGTKCLRREAPRWDAPLRDPALRQLL

SEQ ID NO: 15 - protein, 551 aa, synthetic construct
  source 1..551: note = Signal peptide_Siltuximab heavy chain_Linker_Domain 7 and unstructured C-terminus of PGRN_fusion protein
MYRMQLLSCIALSLALVTNSEVQLVESGGKLLKPGGSLKLSCAASGFTFSSFAMSWFRQSPEKRLEWVAEISSGGSYTYYPDTVTGRFTISRDNAKNTLYLEMSSLRSEDTAMYYCARGLWGYYALDYWGQGTSVTVSSASTKGPSVFPLAPSSKSTSGGTAALGCLVKDYFPEPVTVSWNSGALTSGVHTFPAVLQSSGLYSLSSVVTVPSSSLGTQTYICNVNHKPSNTKVDKKVEPKSCDKTHTCPPCPAPELLGGPSVFLFPPKPKDTLMISRTPEVTCVVVDVSHEDPEVKFNWYVDGVEVHNAKTKPREEQYNSTYRVVSVLTVLHQDWLNGKEYKCKVSNKALPAPIEKTISKAKGQPREPQVYTLPPSRDELTKNQVSLTCLVKGFYPSDIAVEWESNGQPENNYKTTPPVLDSDGSFFLYSKLTVDKSRWQQGNVFSCSVMHEALHNHYTQKSLSLSPGKGSGSGSDVECGEGHFCHDNQTCCRDNRQGWACCPYRQGVCCADRRHCCPAGFRCAARGTKCLRREAPRWDAPLRDPALRQLL